European Patent Specification EP 4 175 718 B1, published October 2, 2024. Title: INDOLE DERIVATIVES AND USES THEREOF FOR TREATING A CANCER. Applicant: UNIVERSITE CLAUDE BERNARD LYON 1 et al. The sequence listing filed with the application follows.

SEQUENCE LISTING (2 sequences)

SEQ ID NO: 1 - protein, 12 aa, artificial
  CK2 peptide substrate
RRREDEESDDEE

SEQ ID NO: 2 - protein, 22 aa, artificial
  CK2 peptide substrate
MSGDEMIFDPTMSKKKKKKKKP